European Patent Application EP 4 509 143 A2, published February 19, 2025. Title: CD38 ANTOBODY DRUG CONJUGATE. Applicant: Sorrento Therapeutics, Inc. Application EP 18746292.4, filed June 20, 2018. The sequence listing filed with the application follows.

SEQUENCE LISTING (3 sequences)

SEQ ID NO: 1 - protein, 118 aa, Homo sapiens
QVQLVESGGGLVKPGGSLRLSCAASGFTFSDDYMSWIRQAPGKGLEWVASVSNGRPTTYYADSVRGRFTISRDNAKNSLYLQMNSLRAEDTAVYYCAREDWGGEFTDWGRGTLVTVSS

SEQ ID NO: 2 - protein, 110 aa, Homo sapiens
QAGLTQPPSASGTSGQRVTISCSGSSSNIGINFVYWYQHLPGTAPKLLIYKNNQRPSGVPDRFSGSKSGNSASLAISGLRSEDEADYYCAAWDDSLSGYVFGSGTKVTVL

SEQ ID NO: 3 - protein, 110 aa, Homo sapiens
QSVLTQPPSASGTSGQRVTISCSGSSSNIGINFVYWYQHLPGTAPKLLIYKNNQRPSGVPDRFSGSKSGNSASLAISGLRSEDEADYYCAAWDDSLSGYVFGSGTKVTVL